European Patent Specification EP 3 843 757 B1, published April 24, 2024. Title: Cryopreserved NK cells preloaded with an antibody construct. Applicant: Affimed GmbH. The sequence listing filed with the application follows.

SEQUENCE LISTING (178 sequences)

SEQ ID NO: 1 - protein, 6 aa, Artificial Sequence
  linker
GGSGGS

SEQ ID NO: 2 - protein, 18 aa, Artificial Sequence
  linker
GGSGGSGGSGGSGGSGGS

SEQ ID NO: 3 - protein, 21 aa, Artificial Sequence
  linker
GGSGGSGGSGGSGGSGGSGGS

SEQ ID NO: 4 - protein, 9 aa, Artificial Sequence
  linker
GGSGGSGGS

SEQ ID NO: 5 - protein, 5 aa, Artificial Sequence
  linker
GGGGS

SEQ ID NO: 6 - protein, 10 aa, Artificial Sequence
  linker
GGGGSGGGGS

SEQ ID NO: 7 - protein, 20 aa, Artificial Sequence
  linker
GGGGSGGGGSGGGGSGGGGS

SEQ ID NO: 8 - protein, 30 aa, Artificial Sequence
  linker
GGGGSGGGGSGGGGSGGGGSGGGGSGGGGS

SEQ ID NO: 9 - protein, 15 aa, Artificial Sequence
  hinge
EPKSCDKTHTCPPCP

SEQ ID NO: 10 - protein, 10 aa, Artificial Sequence
  hinge
DKTHTCPPCP

SEQ ID NO: 11 - protein, 328 aa, Artificial Sequence
  heavy chain constant domain
ASTKGPSVFPLAPSSKSTSGGTAALGCLVKDYFPEPVTVSWNSGALTSGVHTFPAVLQSSGLYSLSSVVVPSSSLGTQTYICNVNHKPSNTKVDKKVEPKSCDKTHTCPPCPAPEFEGGPSVFLFPPKPKDTLMISRTPEVTCVVVAVSHEDPEVKFNWYVDGVEVHNAKTKPREEQYNSTYRVVSVLTVLHQDWLNGKEYKCKVSNKALPAPIEKTISKAKGQPREPQVYTLPPSREEMTKNQVSLTCLVKGFYPSDIAVEWESNGQPENNYKTTPPVLDSDGSFFLYSKLTVDKSRWQQGNVFSCSVMHEALHNHYTQKSLSLSPG

SEQ ID NO: 12 - protein, 328 aa, Homo sapiens
  heavy chain constant domain
ASTKGPSVFPLAPSSKSTSGGTAALGCLVKDYFPEPVTVSWNSGALTSGVHTFPAVLQSSGLYSLSSVVVPSSSLGTQTYICNVNHKPSNTKVDKKVEPKSCDKTHTCPPCPAPELLGGPSVFLFPPKPKDTLMISRTPEVTCVVVDVSHEDPEVKFNWYVDGVEVHNAKTKPREEQYNSTYRVVSVLTVLHQDWLNGKEYKCKVSNKALPAPIEKTISKAKGQPREPQVYTLPPSREEMTKNQVSLTCLVKGFYPSDIAVEWESNGQPENNYKTTPPVLDSDGSFFLYSKLTVDKSRWQQGNVFSCSVMHEALHNHYTQKSLSLSPG

SEQ ID NO: 13 - protein, 106 aa, Homo sapiens
  light chain constant domain
GQPKAAPSVTLFPPSSEELQANKATLVCLISDFYPGAVTVAWKADSSPVKAGVETTTPSKQSNNKYAASSYLSLTPEQWKSHRSYSCQVTHEGSTVEKTVAPTECS

SEQ ID NO: 14 - protein, 107 aa, Homo sapiens [sequence omitted]

SEQ ID NO: 15 - protein, 216 aa, Artificial Sequence
  CH2-CH3 constant domain
APEFEGGPSVFLFPPKPKDTLMISRTPEVTCVVVAVSHEDPEVKFNWYVDGVEVHNAKTKPREEQYNSTYRVVSVLTVLHQDWLNGKEYKCKVSNKALPAPIEKTISKAKGQPREPQVYTLPPSREEMTKNQVSLTCLVKGFYPSDIAVEWESNGQPENNYKTTPPVLDSDGSFFLYSKLTVDKSRWQQGNVFSCSVMHEALHNHYTQKSLSLSPG

SEQ ID NO: 16 - protein, 215 aa, Artificial Sequence
  CH2-CH3 constant domain
APEFEGGPSVFLFPPKPKDTLMISRTPEVTCVVVAVSHEDPEVKFNWYVDGVEVHNAKTKPREEQYNSTYRVVSVLTVLHQDWLNGKEYKCKVSNKALPAPIEKTISKAKGQPREPQVYTKPPSRDELTKNQVSLSCLVKGFYPSDIAVEWESNGQPENNYKTTVPVLDSDGSFRLASYLTVDKSRWQQGNVFSCSVMHEALHNHYTQKSLSLSP

SEQ ID NO: 17 - protein, 216 aa, Artificial Sequence
  ch2-ch3 constant domain
APEFEGGPSVFLFPPKPKDTLMISRTPEVTCVVVAVSHEDPEVKFNWYVDGVEVHNAKTKPREEQYNSTYRVVSVLTVLHQDWLNGKEYKCKVSNKALPAPIEKTISKAKGQPREPQVYTLPPSREEMTKNQVSLYCLVKGFYPSDIAVEWESNGQPENNYKTTPPVLDSDGSFFLYSKLTVDKSRWQQGNVFSCSVMHEALHNHYTQKSLSLSPG

SEQ ID NO: 18 - protein, 216 aa, Artificial Sequence
  ch2-ch3 constant domain
APEFEGGPSVFLFPPKPKDTLMISRTPEVTCVVVAVSHEDPEVKFNWYVDGVEVHNAKTKPREEQYNSTYRVVSVLTVLHQDWLNGKEYKCKVSNKALPAPIEKTISKAKGQPREPQVYTLPPSREEMTKNQVSLTCLVKGFYPSDIAVEWESNGQPENNYKTTPPVLDSDGSFFLTSKLTVDKSRWQQGNVFSCSVMHEALHNHYTQKSLSLSPG

SEQ ID NO: 19 - protein, 98 aa, Homo sapiens
  ch1 domain
ASTKGPSVFPLAPSSKSTSGGTAALGCLVKDYFPEPVTVSWNSGALTSGVHTFPAVLQSSGLYSLSSVVTVPSSSLGTQTYICNVNHKPSNTKVDKKV

SEQ ID NO: 20 - protein, 106 aa, Artificial Sequence
  cl domain
GQPKAAPSVTLFPPSSEELQANKATLVCLISDFYPGAVTVAWKADSSPVKAGVETTTPSKQSNNKYAASSYLSLTPEQWKSHRSYSCQVTHEGSTVEKTVAPTESS

SEQ ID NO: 21 - protein, 107 aa, Artificial Sequence
  cl domain
RTVAAPSVFIFPPSDEQLKSGTASVVCLLNNFYPREAKVQWKVDNALQSGNSQESVTEQDSKDSTYSLSSTLTLSKADYEKHKVYACEVTHQGLSSPVTKSFNRGES

SEQ ID NO: 22 - protein, 216 aa, Homo sapiens
  ch2-ch3 domain
APELLGGPSVFLFPPKPKDTLMISRTPEVTCVVVDVSHEDPEVKFNWYVDGVEVHNAKTKPREEQYNSTYRVVSVLTVLHQDWLNGKEYKCKVSNKALPAPIEKTISKAKGQPREPQVYTLPPSREEMTKNQVSLTCLVKGFYPSDIAVEWESNGQPENNYKTTPPVLDSDGSFFLYSKLTVDKSRWQQGNVFSCSVMHEALHNHYTQKSLSLSPG

SEQ ID NO: 23 - protein, 192 aa, Homo sapiens
  CD16a
GMRTEDLPKAVVFLEPQWYRVLEKDSVTLKCQGAYSPEDNSTQWFHNESLISSQASSYFIDAATVDDSGEYRCQTNLSTLSDPVQLEVHIGWLLLQAPRWVFKEEDPIHLRCHSWKNTALHKVTYLQNGKGRKYFHHNSDFYIPKATLKDSGSYFCRGLFGSKNVSSETVNITITQGLAVSTISSFFPPGYQ

SEQ ID NO: 24 - protein, 192 aa, Cynomolgus
  CD16a
GMRAEDLPKAVVFLEPQWYRVLEKDRVTLKCQGAYSPEDNSTRWFHNESLISSQTSSYFIAAARVNNSGEYRCQTSLSTLSDPVQLEVHIGWLLLQAPRWVFKEEESIHLRCHSWKNTLLHKVTYLQNGKGRKYFHQNSDFYIPKATLKDSGSYFCRGLIGSKNVSSETVNITITQDLAVSSISSFFPPGYQ

SEQ ID NO: 25 - protein, 6 aa, Artificial Sequence
  peptide tag
HHHHHH

SEQ ID NO: 26 - protein, 4 aa, Artificial Sequence
  peptide tag
EPEA

SEQ ID NO: 27 - protein, 121 aa, Artificial Sequence
  variable domain
EVQLLESGGGLVQPGGSLRLSCAVSGIDLSNYAINWVRQAPGKGLEWIGIIWASGTTFYATWAKGRFTISRDNSKNTVYLQMNSLRAEDTAVYYCARTVPGYSTAPYFDLWGQGTLVTVSS

SEQ ID NO: 28 - protein, 110 aa, Artificial Sequence
  variable domain
DIQMTQSPSSVSASVGDRVTITCQSSPSVWSNFLSWYQQKPGKAPKLLIYEASKLTSGVPSRFSGSGSGTDFTLTISSLQPEDFATYYCGGGYSSISDTTFGGGTKVEIK

SEQ ID NO: 29 - protein, 8 aa, Artificial Sequence
  cdr
GYTFTSYY

SEQ ID NO: 30 - protein, 8 aa, Artificial Sequence
  cdr
INPSGGST

SEQ ID NO: 31 - protein, 13 aa, Artificial Sequence
  cdr
ARGSAYYYDFADY

SEQ ID NO: 32 - protein, 6 aa, Artificial Sequence
  cdr
NIGSKN

SEQ ID NO: 33 - skipped

SEQ ID NO: 34 - protein, 9 aa, Artificial Sequence
  cdr
QVWDNYSVL

SEQ ID NO: 35 - protein, 120 aa, Artificial Sequence
  variable domain
QVQLVQSGAEVKKPGESLKVSCKASGYTFTSYYMHWVRQAPGQGLEWMGIINPSGGSTSYAQKFQGRVTMTRDTSTSTVYMELSSLRSEDTAVYYCARGSAYYYDFADYWGQGTLVTVSS

SEQ ID NO: 36 - protein, 106 aa, Artificial Sequence
  variable domain
SYVLTQPSSVSVAPGQTATISCGGHNIGSKNVHWYQQRPGQSPVLVIYQDNKRPSGIPERFSGSNSGNTATLTISGTQAMDEADYYCQVWDNYSVLFGGGTKLTVL

SEQ ID NO: 37 - protein, 255 aa, Artificial Sequence
  scFv
QVQLVQSGAEVKKPGESLKVSCKASGYTFTSYYMHWVRQAPGQGLEWMGIINPSGGSTSYAQKFQGRVTMTRDTSTSTVYMELSSLRSEDTAVYYCARGSAYYYDFADYWGQGTLVTVSSGGSGGSGGSGGSGGSGGSSYVLTQPSSVSVAPGQTATISCGGHNIGSKNVHWYQQRPGQSPVLVIYQDNKRPSGIPERFSGSNSGNTATLTISGTQAMDEADYYCQVWDNYSVLFGGGTKLTVLAAAGSHHHHHH

SEQ ID NO: 38 - protein, 218 aa, Artificial Sequence
  Fab VH
QVQLVQSGAEVKKPGESLKVSCKASGYTFTSYYMHWVRQAPGQGLEWMGIINPSGGSTSYAQKFQGRVTMTRDTSTSTVYMELSSLRSEDTAVYYCARGSAYYYDFADYWGQGTLVTVSSASTKGPSVFPLAPSSKSTSGGTAALGCLVKDYFPEPVTVSWNSGALTSGVHTFPAVLQSSGLYSLSSVVTVPSSSLGTQTYICNVNHKPSNTKVDKKV

SEQ ID NO: 39 - protein, 212 aa, Artificial Sequence
  Fab VL
SYVLTQPSSVSVAPGQTATISCGGHNIGSKNVHWYQQRPGQSPVLVIYQDNKRPSGIPERFSGSNSGNTATLTISGTQAMDEADYYCQVWDNYSVLFGGGTKLTVLGQPKAAPSVTLFPPSSEELQANKATLVCLISDFYPGAVTVAWKADSSPVKAGVETTTPSKQSNNKYAASSYLSLTPEQWKSHRSYSCQVTHEGSTVEKTVAPTECS

SEQ ID NO: 40 - protein, 8 aa, Artificial Sequence
  cdr
GYTFTSYY

SEQ ID NO: 41 - protein, 8 aa, Artificial Sequence
  cdr
IEPMYGST

SEQ ID NO: 42 - protein, 13 aa, Artificial Sequence
  cdr
ARGSAYYYDFADY

SEQ ID NO: 43 - protein, 6 aa, Artificial Sequence
  cdr
NIGSKN

SEQ ID NO: 44 - skipped

SEQ ID NO: 45 - protein, 9 aa, Artificial Sequence
  cdr
QVWDNYSVL

SEQ ID NO: 46 - protein, 120 aa, Artificial Sequence
  variable domain
QVQLVQSGAEVKKPGESLKVSCKASGYTFTSYYMHWVRQAPGQGLEWMGAIEPMYGSTSYAQKFQGRVTMTRDTSTSTVYMELSSLRSEDTAVYYCARGSAYYYDFADYWGQGTLVTVSS

SEQ ID NO: 47 - protein, 106 aa, Artificial Sequence; identical to SEQ ID NO: 36
  variable domain

SEQ ID NO: 48 - protein, 255 aa, Artificial Sequence
  scFv
QVQLVQSGAEVKKPGESLKVSCKASGYTFTSYYMHWVRQAPGQGLEWMGAIEPMYGSTSYAQKFQGRVTMTRDTSTSTVYMELSSLRSEDTAVYYCARGSAYYYDFADYWGQGTLVTVSSGGSGGSGGSGGSGGSGGSSYVLTQPSSVSVAPGQTATISCGGHNIGSKNVHWYQQRPGQSPVLVIYQDNKRPSGIPERFSGSNSGNTATLTISGTQAMDEADYYCQVWDNYSVLFGGGTKLTVLAAAGSHHHHHH

SEQ ID NO: 49 - protein, 218 aa, Artificial Sequence
  Fab VH
QVQLVQSGAEVKKPGESLKVSCKASGYTFTSYYMHWVRQAPGQGLEWMGAIEPMYGSTSYAQKFQGRVTMTRDTSTSTVYMELSSLRSEDTAVYYCARGSAYYYDFADYWGQGTLVTVSSASTKGPSVFPLAPSSKSTSGGTAALGCLVKDYFPEPVTVSWNSGALTSGVHTFPAVLQSSGLYSLSSVVTVPSSSLGTQTYICNVNHKPSNTKVDKKV

SEQ ID NO: 50 - protein, 212 aa, Artificial Sequence; identical to SEQ ID NO: 39
  Fab VL

SEQ ID NO: 51 - protein, 8 aa, Artificial Sequence
  cdr
GYTFTNYY

SEQ ID NO: 52 - protein, 8 aa, Artificial Sequence
  cdr
INPGGGST

SEQ ID NO: 53 - protein, 13 aa, Artificial Sequence
  cdr
ARGSAYYYDFADY

SEQ ID NO: 54 - protein, 6 aa, Artificial Sequence
  cdr
NIGSQS

SEQ ID NO: 55 - skipped

SEQ ID NO: 56 - protein, 9 aa, Artificial Sequence
  cdr
QVWDNYSVV

SEQ ID NO: 57 - protein, 120 aa, Artificial Sequence
  variable domain
QVQLVQSGAEVKKPGESLKVSCKASGYTFTNYYMQWVRQAPGQGLEWMGVINPGGGSTSYAQKFQGRVTMTRDTSTSTVYMELSSLRSEDTAVYYCARGSAYYYDFADYWGQGTLVTVSS

SEQ ID NO: 58 - protein, 106 aa, Artificial Sequence
  variable domain
SYVLTQPSSVSVAPGQTARITCGGHNIGSQSVHWYQQKPGQAPVLVIYQDSKRPSGIPERFSGSNSGNTATLTISGTQAMDEADYYCQVWDNYSVVFGGGTKLTVL

SEQ ID NO: 59 - protein, 255 aa, Artificial Sequence
  scFv
QVQLVQSGAEVKKPGESLKVSCKASGYTFTNYYMQWVRQAPGQGLEWMGVINPGGGSTSYAQKFQGRVTMTRDTSTSTVYMELSSLRSEDTAVYYCARGSAYYYDFADYWGQGTLVTVSSGGSGGSGGSGGSGGSGGSSYVLTQPSSVSVAPGQTARITCGGHNIGSQSVHWYQQKPGQAPVLVIYQDSKRPSGIPERFSGSNSGNTATLTISGTQAMDEADYYCQVWDNYSVVFGGGTKLTVLAAAGSHHHHHH

SEQ ID NO: 60 - protein, 218 aa, Artificial Sequence
  Fab VH
QVQLVQSGAEVKKPGESLKVSCKASGYTFTNYYMQWVRQAPGQGLEWMGVINPGGGSTSYAQKFQGRVTMTRDTSTSTVYMELSSLRSEDTAVYYCARGSAYYYDFADYWGQGTLVTVSSASTKGPSVFPLAPSSKSTSGGTAALGCLVKDYFPEPVTVSWNSGALTSGVHTFPAVLQSSGLYSLSSVVTVPSSSLGTQTYICNVNHKPSNTKVDKKV

SEQ ID NO: 61 - protein, 212 aa, Artificial Sequence
  Fab VL
SYVLTQPSSVSVAPGQTARITCGGHNIGSQSVHWYQQKPGQAPVLVIYQDSKRPSGIPERFSGSNSGNTATLTISGTQAMDEADYYCQVWDNYSVVFGGGTKLTVLGQPKAAPSVTLFPPSSEELQANKATLVCLISDFYPGAVTVAWKADSSPVKAGVETTTPSKQSNNKYAASSYLSLTPEQWKSHRSYSCQVTHEGSTVEKTVAPTECS

SEQ ID NO: 62 - protein, 8 aa, Artificial Sequence
  cdr
GYSFSDFY

SEQ ID NO: 63 - protein, 8 aa, Artificial Sequence
  cdr
INPGGAST

SEQ ID NO: 64 - protein, 13 aa, Artificial Sequence
  cdr
ARGSAYYYDFADY

SEQ ID NO: 65 - protein, 6 aa, Artificial Sequence
  cdr
NIGRQS

SEQ ID NO: 66 - skipped

SEQ ID NO: 67 - protein, 9 aa, Artificial Sequence
  cdr
QVWDNYTVV

SEQ ID NO: 68 - protein, 120 aa, Artificial Sequence
  variable domain
QVQLVQSGAEVKKPGESLKVSCKASGYSFSDFYIQWVRQAPGQGLEWMGIINPGGASTTYAQKFQGRVTMTRDTSTSTVYMELSSLRSEDTAVYYCARGSAYYYDFADYWGQGTLVTVSS

SEQ ID NO: 69 - protein, 106 aa, Artificial Sequence
  variable domain
SYVLTQPSSVSVAPGQTARITCGGYNIGRQSVHWYQQKPGQAPVLVIYQDSKRPSGIPERFSGSNSGNTATLTISGTQAMDEADYYCQVWDNYTVVFGGGTKLTVL

SEQ ID NO: 70 - protein, 255 aa, Artificial Sequence
  scFv
QVQLVQSGAEVKKPGESLKVSCKASGYSFSDFYIQWVRQAPGQGLEWMGIINPGGASTTYAQKFQGRVTMTRDTSTSTVYMELSSLRSEDTAVYYCARGSAYYYDFADYWGQGTLVTVSSGGSGGSGGSGGSGGSGGSSYVLTQPSSVSVAPGQTARITCGGYNIGRQSVHWYQQKPGQAPVLVIYQDSKRPSGIPERFSGSNSGNTATLTISGTQAMDEADYYCQVWDNYTVVFGGGTKLTVLAAAGSHHHHHH

SEQ ID NO: 71 - protein, 218 aa, Artificial Sequence
  Fab VH
QVQLVQSGAEVKKPGESLKVSCKASGYSFSDFYIQWVRQAPGQGLEWMGIINPGGASTTYAQKFQGRVTMTRDTSTSTVYMELSSLRSEDTAVYYCARGSAYYYDFADYWGQGTLVTVSSASTKGPSVFPLAPSSKSTSGGTAALGCLVKDYFPEPVTVSWNSGALTSGVHTFPAVLQSSGLYSLSSVVTVPSSSLGTQTYICNVNHKPSNTKVDKKV

SEQ ID NO: 72 - protein, 212 aa, Artificial Sequence
  Fab VL
SYVLTQPSSVSVAPGQTARITCGGYNIGRQSVHWYQQKPGQAPVLVIYQDSKRPSGIPERFSGSNSGNTATLTISGTQAMDEADYYCQVWDNYTVVFGGGTKLTVLGQPKAAPSVTLFPPSSEELQANKATLVCLISDFYPGAVTVAWKADSSPVKAGVETTTPSKQSNNKYAASSYLSLTPEQWKSHRSYSCQVTHEGSTVEKTVAPTECS

SEQ ID NO: 73 - protein, 8 aa, Artificial Sequence
  cdr
GYTFSSYY

SEQ ID NO: 74 - protein, 8 aa, Artificial Sequence
  cdr
IEPRGVRI

SEQ ID NO: 75 - protein, 13 aa, Artificial Sequence
  cdr
ARGSAYYYDFADY

SEQ ID NO: 76 - protein, 6 aa, Artificial Sequence
  cdr
NIGSTN

SEQ ID NO: 77 - skipped

SEQ ID NO: 78 - protein, 9 aa, Artificial Sequence
  cdr
QVWDNYSVQ

SEQ ID NO: 79 - protein, 120 aa, Artificial Sequence
  variable domain
QVQLVQSGAEVKKPGESLKVSCKASGYTFSSYYMHWVRQAPGQGLEWMGAIEPRGVRISYAQKFQGRVTMTRDTSTSTVYMELSSLRSEDTAVYYCARGSAYYYDFADYWGQGTLVTVSS

SEQ ID NO: 80 - protein, 106 aa, Artificial Sequence
  variable domain
SYVLTQPSSVSVAPGQTARITCGGHNIGSTNVHWYQQKPGQAPVLVIYQDSKRPSGIPERFSGSNSGNTATLTISGTQAMDEADYYCQVWDNYSVQFGGGTKLTVL

SEQ ID NO: 81 - protein, 255 aa, Artificial Sequence
  scFv
QVQLVQSGAEVKKPGESLKVSCKASGYTFSSYYMHWVRQAPGQGLEWMGAIEPRGVRISYAQKFQGRVTMTRDTSTSTVYMELSSLRSEDTAVYYCARGSAYYYDFADYWGQGTLVTVSSGGSGGSGGSGGSGGSGGSSYVLTQPSSVSVAPGQTARITCGGHNIGSTNVHWYQQKPGQAPVLVIYQDSKRPSGIPERFSGSNSGNTATLTISGTQAMDEADYYCQVWDNYSVQFGGGTKLTVLAAAGSHHHHHH

SEQ ID NO: 82 - protein, 218 aa, Artificial Sequence
  Fab VH
QVQLVQSGAEVKKPGESLKVSCKASGYTFSSYYMHWVRQAPGQGLEWMGAIEPRGVRISYAQKFQGRVTMTRDTSTSTVYMELSSLRSEDTAVYYCARGSAYYYDFADYWGQGTLVTVSSASTKGPSVFPLAPSSKSTSGGTAALGCLVKDYFPEPVTVSWNSGALTSGVHTFPAVLQSSGLYSLSSVVTVPSSSLGTQTYICNVNHKPSNTKVDKKV

SEQ ID NO: 83 - protein, 212 aa, Artificial Sequence
  Fab VL
SYVLTQPSSVSVAPGQTARITCGGHNIGSTNVHWYQQKPGQAPVLVIYQDSKRPSGIPERFSGSNSGNTATLTISGTQAMDEADYYCQVWDNYSVQFGGGTKLTVLGQPKAAPSVTLFPPSSEELQANKATLVCLISDFYPGAVTVAWKADSSPVKAGVETTTPSKQSNNKYAASSYLSLTPEQWKSHRSYSCQVTHEGSTVEKTVAPTECS

SEQ ID NO: 84 - protein, 8 aa, Artificial Sequence
  cdr
GYTFTNYY

SEQ ID NO: 85 - protein, 8 aa, Artificial Sequence
  cdr
INPSGGVT

SEQ ID NO: 86 - protein, 13 aa, Artificial Sequence
  cdr
ARGSAYYYDFADY

SEQ ID NO: 87 - protein, 6 aa, Artificial Sequence
  cdr
NIGSKS

SEQ ID NO: 88 - skipped

SEQ ID NO: 89 - protein, 9 aa, Artificial Sequence
  cdr
QVWDDYIVL

SEQ ID NO: 90 - protein, 120 aa, Artificial Sequence
  variable domain
QVQLVQSGAEVKKPGESLKVSCKASGYTFTNYYMQWVRQAPGQGLEWMGIINPSGGVTSYAQKFQGRVTMTRDTSTSTVYMELSSLRSEDTAVYYCARGSAYYYDFADYWGQGTLVTVSS

SEQ ID NO: 91 - protein, 106 aa, Artificial Sequence
  variable domain
SYVLTQPSSVSVAPGQTARITCGGNNIGSKSVHWYQQKPGQAPVLVIYQDKKRPSGIPERFSGSNSGNTATLTISGTQAMDEADYYCQVWDDYIVLFGGGTKLTVL

SEQ ID NO: 92 - protein, 255 aa, Artificial Sequence
  scFv
QVQLVQSGAEVKKPGESLKVSCKASGYTFTNYYMQWVRQAPGQGLEWMGIINPSGGVTSYAQKFQGRVTMTRDTSTSTVYMELSSLRSEDTAVYYCARGSAYYYDFADYWGQGTLVTVSSGGSGGSGGSGGSGGSGGSSYVLTQPSSVSVAPGQTARITCGGNNIGSKSVHWYQQKPGQAPVLVIYQDKKRPSGIPERFSGSNSGNTATLTISGTQAMDEADYYCQVWDDYIVLFGGGTKLTVLAAAGSHHHHHH

SEQ ID NO: 93 - protein, 218 aa, Artificial Sequence
  Fab VH
QVQLVQSGAEVKKPGESLKVSCKASGYTFTNYYMQWVRQAPGQGLEWMGIINPSGGVTSYAQKFQGRVTMTRDTSTSTVYMELSSLRSEDTAVYYCARGSAYYYDFADYWGQGTLVTVSSASTKGPSVFPLAPSSKSTSGGTAALGCLVKDYFPEPVTVSWNSGALTSGVHTFPAVLQSSGLYSLSSVVTVPSSSLGTQTYICNVNHKPSNTKVDKKV

SEQ ID NO: 94 - protein, 212 aa, Artificial Sequence
  Fab VL
SYVLTQPSSVSVAPGQTARITCGGNNIGSKSVHWYQQKPGQAPVLVIYQDKKRPSGIPERFSGSNSGNTATLTISGTQAMDEADYYCQVWDDYIVLFGGGTKLTVLGQPKAAPSVTLFPPSSEELQANKATLVCLISDFYPGAVTVAWKADSSPVKAGVETTTPSKQSNNKYAASSYLSLTPEQWKSHRSYSCQVTHEGSTVEKTVAPTECS

SEQ ID NO: 95 - protein, 8 aa, Artificial Sequence
  cdr
GYTFTNYY

SEQ ID NO: 96 - protein, 8 aa, Artificial Sequence
  cdr
IEPDGGRR

SEQ ID NO: 97 - protein, 13 aa, Artificial Sequence
  cdr
ARGSAYYYDFADY

SEQ ID NO: 98 - protein, 6 aa, Artificial Sequence
  cdr
QGVSGD

SEQ ID NO: 99 - skipped

SEQ ID NO: 100 - protein, 9 aa, Artificial Sequence
  cdr
QQWDNYSVT

SEQ ID NO: 101 - protein, 120 aa, Artificial Sequence
  variable domain
QVQLVQSGAEVKKPGESLKVSCKASGYTFTNYYMHWVRQAPGQGLEWMGVIEPDGGRRTYAQKFQGRVTMTRDTSTSTVYMELSSLRSEDTAVYYCARGSAYYYDFADYWGQGTLVTVSS

SEQ ID NO: 102 - protein, 107 aa, Artificial Sequence
  variable domain
EIVLTQSPATLSLSPGERATLSCRGHQGVSGDVHWYQQKPGQAPRLLIYQANKRASGIPARFSGSGSGTEFTLTISSLEPEDFAVYYCQQWDNYSVTFGQGTKVEIK

SEQ ID NO: 103 - protein, 256 aa, Artificial Sequence
  scFv
QVQLVQSGAEVKKPGESLKVSCKASGYTFTNYYMHWVRQAPGQGLEWMGVIEPDGGRRTYAQKFQGRVTMTRDTSTSTVYMELSSLRSEDTAVYYCARGSAYYYDFADYWGQGTLVTVSSGGSGGSGGSGGSGGSGGSEIVLTQSPATLSLSPGERATLSCRGHQGVSGDVHWYQQKPGQAPRLLIYQANKRASGIPARFSGSGSGTEFTLTISSLEPEDFAVYYCQQWDNYSVTFGQGTKVEIKAAAGSHHHHHH

SEQ ID NO: 104 - protein, 218 aa, Artificial Sequence
  Fab VH
QVQLVQSGAEVKKPGESLKVSCKASGYTFTNYYMHWVRQAPGQGLEWMGVIEPDGGRRTYAQKFQGRVTMTRDTSTSTVYMELSSLRSEDTAVYYCARGSAYYYDFADYWGQGTLVTVSSASTKGPSVFPLAPSSKSTSGGTAALGCLVKDYFPEPVTVSWNSGALTSGVHTFPAVLQSSGLYSLSSVVTVPSSSLGTQTYICNVNHKPSNTKVDKKV

SEQ ID NO: 105 - protein, 214 aa, Artificial Sequence
  Fab VL
EIVLTQSPATLSLSPGERATLSCRGHQGVSGDVHWYQQKPGQAPRLLIYQANKRASGIPARFSGSGSGTEFTLTISSLEPEDFAVYYCQQWDNYSVTFGQGTKVEIKRTVAAPSVFIFPPSDEQLKSGTASVVCLLNNFYPREAKVQWKVDNALQSGNSQESVTEQDSKDSTYSLSSTLTLSKADYEKHKVYACEVTHQGLSSPVTKSFNRGEC

SEQ ID NO: 106 - protein, 8 aa, Artificial Sequence
  cdr
GFTFSNYD

SEQ ID NO: 107 - protein, 8 aa, Artificial Sequence
  cdr
ISTRGDIT

SEQ ID NO: 108 - protein, 14 aa, Artificial Sequence
  cdr
ARQDYYTDYMGFAY

SEQ ID NO: 109 - protein, 6 aa, Artificial Sequence
  cdr
EDIYNG

SEQ ID NO: 110 - skipped

SEQ ID NO: 111 - protein, 9 aa, Artificial Sequence
  cdr
AGPHKYPLT

SEQ ID NO: 112 - protein, 121 aa, Artificial Sequence
  variable domain
EVQLLESGGGLVQPGGSLRLSCAASGFTFSNYDMAWVRQAPGKGLEWVSSISTRGDITSYRDSVKGRFTISRDNSKNTLYLQMNSLRAEDTAVYYCARQDYYTDYMGFAYWGQGTLVTVSS

SEQ ID NO: 113 - protein, 107 aa, Artificial Sequence
  variable domain
AIQMTQSPSSLSASVGDRVTITCRASEDIYNGLAWYQQKPGKAPKLLIYGASSLQDGVPSRFSGSGSGTEFTLTISSLQPEDEATYYCAGPHKYPLTFGGGTKVEIK

SEQ ID NO: 114 - protein, 254 aa, Artificial Sequence
  scFv
EVQLLESGGGLVQPGGSLRLSCAASGFTFSNYDMAWVRQAPGKGLEWVSSISTRGDITSYRDSVKGRFTISRDNSKNTLYLQMNSLRAEDTAVYYCARQDYYTDYMGFAYWGQGTLVTVSSGGGGSGGGGSGGGGSAIQMTQSPSSLSASVGDRVTITCRASEDIYNGLAWYQQKPGKAPKLLIYGASSLQDGVPSRFSGSGSGTEFTLTISSLQPEDEATYYCAGPHKYPLTFGGGTKVEIKAAAGSHHHHHH

SEQ ID NO: 115 - protein, 218 aa, Artificial Sequence
  Fab VH
EVQLLESGGGLVQPGGSLRLSCAASGFTFSNYDMAWVRQAPGKGLEWVSSISTRGDITSYRDSVKGRFTISRDNSKNTLYLQMNSLRAEDTAVYYCARQDYYTDYMGFAYWGQGTLVTVSSASTKGPSVFPLAPSSKSTSGGTAALGCLVKDYFPEPVTVSWNSGALTSGVHTFPAVLQSSGLYSLSSVVVPSSSLGTQTYICNVNHKPSNTKVDKKV

SEQ ID NO: 116 - protein, 214 aa, Artificial Sequence
  Fab VL
AIQMTQSPSSLSASVGDRVTITCRASEDIYNGLAWYQQKPGKAPKLLIYGASSLQDGVPSRFSGSGSGTEFTLTISSLQPEDEATYYCAGPHKYPLTFGGGTKVEIKRTVAAPSVFIFPPSDEQLKSGTASVVCLLNNFYPREAKVQWKVDNALQSGNSQESVTEQDSKDSTYSLSSTLTLSKADYEKHKVYACEVTHQGLSSPVTKSFNRGEC

SEQ ID NO: 117 - protein, 8 aa, Artificial Sequence
  cdr
GFTFSNFD

SEQ ID NO: 118 - protein, 8 aa, Artificial Sequence
  cdr
ITTGGGDT

SEQ ID NO: 119 - protein, 16 aa, Artificial Sequence
  cdr
VRHGYYDGYHLFDYWG

SEQ ID NO: 120 - protein, 6 aa, Artificial Sequence
  cdr
QGISNN

SEQ ID NO: 121 - skipped

SEQ ID NO: 122 - protein, 9 aa, Artificial Sequence
  cdr
QQFTSLPYT

SEQ ID NO: 123 - protein, 121 aa, Artificial Sequence
  variable domain
EVQLVESGGGLVQPGGSLRLSCAASGFTFSNFDMAWVRQAPGKGLVWVSSITTGGGDTYYADSVKGRFTISRDNAKSTLYLQMDSLRSEDTAVYYCVRHGYYDGYHLFDYWGQGTLVTVSS

SEQ ID NO: 124 - protein, 107 aa, Artificial Sequence
  variable domain
DIQMTQSPSSLSASVGDRVTITCRANQGISNNLNWYQQKPGKAPKPLIYYTSNLQSGVPSRFSGSGSGTDYTLTISSLQPEDFATYYCQQFTSLPYTFGQGTKLEIK

SEQ ID NO: 125 - protein, 254 aa, Artificial Sequence
  scFv
EVQLVESGGGLVQPGGSLRLSCAASGFTFSNFDMAWVRQAPGKGLVWVSSITTGGGDTYYADSVKGRFTISRDNAKSTLYLQMDSLRSEDTAVYYCVRHGYYDGYHLFDYWGQGTLVTVSSGGGGSGGGGSGGGGSDIQMTQSPSSLSASVGDRVTITCRANQGISNNLNWYQQKPGKAPKPLIYYTSNLQSGVPSRFSGSGSGTDYTLTISSLQPEDFATYYCQQFTSLPYTFGQGTKLEIKAAAGSHHHHHH

SEQ ID NO: 126 - protein, 218 aa, Artificial Sequence
  Fab VH
EVQLVESGGGLVQPGGSLRLSCAASGFTFSNFDMAWVRQAPGKGLVWVSSITTGGGDTYYADSVKGRFTISRDNAKSTLYLQMDSLRSEDTAVYYCVRHGYYDGYHLFDYWGQGTLVTVSSASTKGPSVFPLAPSSKSTSGGTAALGCLVKDYFPEPVTVSWNSGALTSGVHTFPAVLQSSGLYSLSSVVVPSSSLGTQTYICNVNHKPSNTKVDKKV

SEQ ID NO: 127 - protein, 214 aa, Artificial Sequence
  Fab VL
DIQMTQSPSSLSASVGDRVTITCRANQGISNNLNWYQQKPGKAPKPLIYYTSNLQSGVPSRFSGSGSGTDYTLTISSLQPEDFATYYCQQFTSLPYTFGQGTKLEIKRTVAAPSVFIFPPSDEQLKSGTASVVCLLNNFYPREAKVQWKVDNALQSGNSQESVTEQDSKDSTYSLSSTLTLSKADYEKHKVYACEVTHQGLSSPVTKSFNRGEC

SEQ ID NO: 128 - protein, 9 aa, Artificial Sequence
  cdr
GSVSSGSYY

SEQ ID NO: 129 - protein, 7 aa, Artificial Sequence
  cdr
IYYSGST

SEQ ID NO: 130 - protein, 12 aa, Artificial Sequence
  cdr
ARNPISIPAFDI

SEQ ID NO: 131 - protein, 6 aa, Artificial Sequence
  cdr
NIGSKS

SEQ ID NO: 132 - skipped

SEQ ID NO: 133 - protein, 11 aa, Artificial Sequence
  cdr
QVWDTSSDHVL

SEQ ID NO: 134 - protein, 120 aa, Artificial Sequence
  variable domain
QVQLQESGPGLVKPSETLSLTCTVSGGSVSSGSYYWSWIRQPPGKGLEWIGYIYYSGSTNYNPSLKSRVTISVDTSKNQFSLKLSSVTAADTAVYYCARNPISIPAFDIWGQGTMVTVSS

SEQ ID NO: 135 - protein, 108 aa, Artificial Sequence
  variable domain
QPVLTQPPSVSVAPGKTARITCGGNNIGSKSVHWYQQKPGQAPVLVIYYDSDRPSGIPERFSGSNSGNTATLTISRVEAGDEADYYCQVWDTSSDHVLFGGGTKLTVL

SEQ ID NO: 136 - protein, 257 aa, Artificial Sequence
  scFv
QVQLQESGPGLVKPSETLSLTCTVSGGSVSSGSYYWSWIRQPPGKGLEWIGYIYYSGSTNYNPSLKSRVTISVDTSKNQFSLKLSSVTAADTAVYYCARNPISIPAFDIWGQGTMVTVSSGGSGGSGGSGGSGGSGGSQPVLTQPPSVSVAPGKTARITCGGNNIGSKSVHWYQQKPGQAPVLVIYYDSDRPSGIPERFSGSNSGNTATLTISRVEAGDEADYYCQVWDTSSDHVLFGGGTKLTVLAAAGSHHHHHH

SEQ ID NO: 137 - protein, 217 aa, Artificial Sequence
  Fab VH
QVQLQESGPGLVKPSETLSLTCTVSGGSVSSGSYYWSWIRQPPGKGLEWIGYIYYSGSTNYNPSLKSRVTISVDTSKNQFSLKLSSVTAADTAVYYCARNPISIPAFDIWGQGTMVTVSSASTKGPSVFPLAPSSKSTSGGTAALGCLVKDYFPEPVTVSWNSGALTSGVHTFPAVLQSSGLYSLSSVVVPSSSLGTQTYICNVNHKPSNTKVDKKV

SEQ ID NO: 138 - protein, 214 aa, Artificial Sequence
  Fab VL
QPVLTQPPSVSVAPGKTARITCGGNNIGSKSVHWYQQKPGQAPVLVIYYDSDRPSGIPERFSGSNSGNTATLTISRVEAGDEADYYCQVWDTSSDHVLFGGGTKLTVLGQPKAAPSVTLFPPSSEELQANKATLVCLISDFYPGAVTVAWKADSSPVKAGVETTTPSKQSNNKYAASSYLSLTPEQWKSHRSYSCQVTHEGSTVEKTVAPTECS

SEQ ID NO: 139 - protein, 8 aa, Artificial Sequence
  cdr
GYMFSTFW

SEQ ID NO: 140 - protein, 8 aa, Artificial Sequence
  cdr
IYPGDSNT

SEQ ID NO: 141 - protein, 14 aa, Artificial Sequence
  cdr
AKIRDGYSYDAFDL

SEQ ID NO: 142 - protein, 9 aa, Artificial Sequence
  cdr
SSDVGGYNY

SEQ ID NO: 143 - skipped

SEQ ID NO: 144 - protein, 12 aa, Artificial Sequence
  cdr
SSYTSSSTLAYV

SEQ ID NO: 145 - protein, 121 aa, Artificial Sequence
  variable domain
QVQLVQSGAEAKKPGESLRISCRASGYMFSTFWIGWVRQMPGKGLEWVASIYPGDSNTIYSPSFQGQVTISADKSINTTYLQWSGLKASDTATYYCAKIRDGYSYDAFDLWGQGTMVTVSS

SEQ ID NO: 146 - protein, 112 aa, Artificial Sequence
  variable domain
QSALTQPASVSGSPGQSITISCTGTSSDVGGYNYVSWYQQHPGKAPKLMIYDVSNRPSGVSNRFSGSKSGNTASLTISGLQAEDEADYYCSSYTSSSTLAYVFGTGTKLTVL

SEQ ID NO: 147 - protein, 262 aa, Artificial Sequence
  scFv
QVQLVQSGAEAKKPGESLRISCRASGYMFSTFWIGWVRQMPGKGLEWVASIYPGDSNTIYSPSFQGQVTISADKSINTTYLQWSGLKASDTATYYCAKIRDGYSYDAFDLWGQGTMVTVSSGGSGGSGGSGGSGGSGGSQSALTQPASVSGSPGQSITISCTGTSSDVGGYNYVSWYQQHPGKAPKLMIYDVSNRPSGVSNRFSGSKSGNTASLTISGLQAEDEADYYCSSYTSSSTLAYVFGTGTKLTVLAAAGSHHHHHH

SEQ ID NO: 148 - protein, 218 aa, Artificial Sequence
  Fab VH
QVQLVQSGAEAKKPGESLRISCRASGYMFSTFWIGWVRQMPGKGLEWVASIYPGDSNTIYSPSFQGQVTISADKSINTTYLQWSGLKASDTATYYCAKIRDGYSYDAFDLWGQGTMVTVSSASTKGPSVFPLAPSSKSTSGGTAALGCLVKDYFPEPVTVSWNSGALTSGVHTFPAVLQSSGLYSLSSVVVPSSSLGTQTYICNVNHKPSNTKVDKKV

SEQ ID NO: 149 - protein, 218 aa, Artificial Sequence
  Fab VL
QSALTQPASVSGSPGQSITISCTGTSSDVGGYNYVSWYQQHPGKAPKLMIYDVSNRPSGVSNRFSGSKSGNTASLTISGLQAEDEADYYCSSYTSSSTLAYVFGTGTKLTVLGQPKAAPSVTLFPPSSEELQANKATLVCLISDFYPGAVTVAWKADSSPVKAGVETTTPSKQSNNKYAASSYLSLTPEQWKSHRSYSCQVTHEGSTVEKTVAPTECS

SEQ ID NO: 150 - protein, 8 aa, Artificial Sequence
  cdr
GFTFSSYA

SEQ ID NO: 151 - protein, 8 aa, Artificial Sequence
  cdr
ISYDGSNK

SEQ ID NO: 152 - protein, 13 aa, Artificial Sequence
  cdr
ARDGGYYHYGLDV

SEQ ID NO: 153 - protein, 6 aa, Artificial Sequence
  cdr
KLGDKY

SEQ ID NO: 154 - skipped

SEQ ID NO: 155 - protein, 9 aa, Artificial Sequence
  cdr
QAWDSSTGV

SEQ ID NO: 156 - protein, 120 aa, Artificial Sequence
  variable domain
EVQLVESGGGVVQPGRSLRLSCAASGFTFSSYAMHWVRQAPGKGLEWVAVISYDGSNKYYADSVKGRFTISRDNSKNTLYLQMNSLRTEDTAVYYCARDGGYYHYGLDVWGQGTTVTVSS

SEQ ID NO: 157 - protein, 106 aa, Artificial Sequence
  variable domain
SYELTQPPSVSVSPGQTASITCSGDKLGDKYASWYQRKPGQSPVLLIYQDAKRPSGIPERFSGSNSGNTATLTISGTQAMDEADYYCQAWDSSTGVFGGGTKLTVL

SEQ ID NO: 158 - protein, 255 aa, Artificial Sequence
  scFv
EVQLVESGGGVVQPGRSLRLSCAASGFTFSSYAMHWVRQAPGKGLEWVAVISYDGSNKYYADSVKGRFTISRDNSKNTLYLQMNSLRTEDTAVYYCARDGGYYHYGLDVWGQGTTVTVSSGGSGGSGGSGGSGGSGGSSYELTQPPSVSVSPGQTASITCSGDKLGDKYASWYQRKPGQSPVLLIYQDAKRPSGIPERFSGSNSGNTATLTISGTQAMDEADYYCQAWDSSTGVFGGGTKLTVLAAAGSHHHHHH

SEQ ID NO: 159 - protein, 217 aa, Artificial Sequence
  Fab VH
EVQLVESGGGVVQPGRSLRLSCAASGFTFSSYAMHWVRQAPGKGLEWVAVISYDGSNKYYADSVKGRFTISRDNSKNTLYLQMNSLRTEDTAVYYCARDGGYYHYGLDVWGQGTTVTVSSASTKGPSVFPLAPSSKSTSGGTAALGCLVKDYFPEPVTVSWNSGALTSGVHTFPAVLQSSGLYSLSSVVVPSSSLGTQTYICNVNHKPSNTKVDKKV

SEQ ID NO: 160 - protein, 212 aa, Artificial Sequence
  Fab VL
SYELTQPPSVSVSPGQTASITCSGDKLGDKYASWYQRKPGQSPVLLIYQDAKRPSGIPERFSGSNSGNTATLTISGTQAMDEADYYCQAWDSSTGVFGGGTKLTVLGQPKAAPSVTLFPPSSEELQANKATLVCLISDFYPGAVTVAWKADSSPVKAGVETTTPSKQSNNKYAASSYLSLTPEQWKSHRSYSCQVTHEGSTVEKTVAPTECS

SEQ ID NO: 161 - protein, 489 aa, Artificial Sequence
  tandem diabody construct
QVQLQESGPGLVKPSETLSLTCTVSGGSVSSGSYYWSWIRQPPGKGLEWIGYIYYSGSTNYNPSLKSRVTISVDTSKNQFSLKLSSVTAADTAVYYCARNPISIPAFDIWGQGTMVTVSSGGSGGSGGSSYVLTQPSSVSVAPGQTATISCGGHNIGSKNVHWYQQRPGQSPVLVIYQDNKRPSGIPERFSGSNSGNTATLTISGTQAMDEADYYCQVWDNYSVLFGGGTKLTVLGGSGGSQVQLVQSGAEVKKPGESLKVSCKASGYTFTSYYMHWVRQAPGQGLEWMGIINPSGGSTSYAQKFQGRVTMTRDTSTSTVYMELSSLRSEDTAVYYCARGSAYYYDFADYWGQGTLVTVSSGGSGGSGGSQPVLTQPPSVSVAPGKTARITCGGNNIGSKSVHWYQQKPGQAPVLVIYYDSDRPSGIPERFSGSNSGNTATLTISRVEAGDEADYYCQVWDTSSDHVLFGGGTKLTVLAAAGSHHHHHH

SEQ ID NO: 162 - protein, 705 aa, Artificial Sequence
  scFv-IgAb polypeptide chain
QVQLVQSGAEVKKPGESLKVSCKASGYTFTSYYMHWVRQAPGQGLEWMGIINPSGGSTSYAQKFQGRVTMTRDTSTSTVYMELSSLRSEDTAVYYCARGSAYYYDFADYWGQGTLVTVSSASTKGPSVFPLAPSSKSTSGGTAALGCLVKDYFPEPVTVSWNSGALTSGVHTFPAVLQSSGLYSLSSVVTVPSSSLGTQTYICNVNHKPSNTKVDKKVEPKSCDKTHTCPPCPAPEFEGGPSVFLFPPKPKDTLMISRTPEVTCVVVAVSHEDPEVKFNWYVDGVEVHNAKTKPREEQYNSTYRVVSVLTVLHQDWLNGKEYKCKVSNKALPAPIEKTISKAKGQPREPQVYTLPPSREEMTKNQVSLTCLVKGFYPSDIAVEWESNGQPENNYKTTPPVLDSDGSFFLYSKLTVDKSRWQQGNVFSCSVMHEALHNHYTQKSLSLSPGGGGGSGGGGSQVQLQESGPGLVKPSETLSLTCTVSGGSVSSGSYYWSWIRQPPGKGLEWIGYIYYSGSTNYNPSLKSRVTISVDTSKNQFSLKLSSVTAADTAVYYCARNPISIPAFDIWGQGTMVTVSSGGSGGSGGSGGSGGSGGSQPVLTQPPSVSVAPGKTARITCGGNNIGSKSVHWYQQKPGQAPVLVIYYDSDRPSGIPERFSGSNSGNTATLTISRVEAGDEADYYCQVWDTSSDHVLFGGGTKLTVL

SEQ ID NO: 163 - protein, 212 aa, Artificial Sequence; identical to SEQ ID NO: 39
  scFv-IgAb polypeptide chain

SEQ ID NO: 164 - protein, 481 aa, Artificial Sequence
  tandem diabody construct
EVQLLESGGGLVQPGGSLRLSCAASGFTFSNYDMAWVRQAPGKGLEWVSSISTRGDITSYRDSVKGRFTISRDNSKNTLYLQMNSLRAEDTAVYYCARQDYYTDYMGFAYWGQGTLVTVSSGGSGGSGGSGGSSYVLTQPSSVSVAPGQTATISCGGHNIGSKNVHWYQQRPGQSPVLVIYQDNKRPSGIPERFSGSNSGNTATLTISGTQAMDEADYYCQVWDNYSVLFGGGTKLTVLGGSQVQLVQSGAEVKKPGESLKVSCKASGYTFTSYYMHWVRQAPGQGLEWMGAIEPMYGSTSYAQKFQGRVTMTRDTSTSTVYMELSSLRSEDTAVYYCARGSAYYYDFADYWGQGTLVTVSSGGSGGSGGSGGSAIQMTQSPSSLSASVGDRVTITCRASEDIYNGLAWYQQKPGKAPKLLIYGASSLQDGVPSRFSGSGSGTEFTLTISSLQPEDEATYYCAGPHKYPLTFGGGTKVEIK

SEQ ID NO: 165 - protein, 727 aa, Artificial Sequence
  scFv-IgAb polypeptide chain
EVQLLESGGGLVQPGGSLRLSCAASGFTFSNYDMAWVRQAPGKGLEWVSSISTRGDITSYRDSVKGRFTISRDNSKNTLYLQMNSLRAEDTAVYYCARQDYYTDYMGFAYWGQGTLVTVSSASTKGPSVFPLAPSSKSTSGGTAALGCLVKDYFPEPVTVSWNSGALTSGVHTFPAVLQSSGLYSLSSVVTVPSSSLGTQTYICNVNHKPSNTKVDKKVEPKSCDKTHTCPPCPAPEFEGGPSVFLFPPKPKDTLMISRTPEVTCVVVAVSHEDPEVKFNWYVDGVEVHNAKTKPREEQYNSTYRVVSVLTVLHQDWLNGKEYKCKVSNKALPAPIEKTISKAKGQPREPQVYTLPPSREEMTKNQVSLTCLVKGFYPSDIAVEWESNGQPENNYKTTPPVLDSDGSFFLYSKLTVDKSRWQQGNVFSCSVMHEALHNHYTQKSLSLSPGGGGGSGGGGSGGGGSGGGGSGGGGSGGGGSSYVLTQPSSVSVAPGQTATISCGGHNIGSKNVHWYQQRPGQSPVLVIYQDNKRPSGIPERFSGSNSGNTATLTISGTQAMDEADYYCQVWDNYSVLFGGGTKLTVLGGSGGSGGSGGSGGSGGSGGSQVQLVQSGAEVKKPGESLKVSCKASGYTFTSYYMHWVRQAPGQGLEWMGAIEPMYGSTSYAQKFQGRVTMTRDTSTSTVYMELSSLRSEDTAVYYCARGSAYYYDFADYWGQGTLVTVSS

SEQ ID NO: 166 - protein, 214 aa, Artificial Sequence; identical to SEQ ID NO: 116
  scFv-IgAb polypeptide chain

SEQ ID NO: 167 - protein, 729 aa, Artificial Sequence
  KiH-scDb-Fc polypeptide chain
DKTHTCPPCPAPEFEGGPSVFLFPPKPKDTLMISRTPEVTCVVVAVSHEDPEVKFNWYVDGVEVHNAKTKPREEQYNSTYRVVSVLTVLHQDWLNGKEYKCKVSNKALPAPIEKTISKAKGQPREPQVYTLPPSREEMTKNQVSLTCLVKGFYPSDIAVEWESNGQPENNYKTTPPVLDSDGSFFLTSKLTVDKSRWQQGNVFSCSVMHEALHNHYTQKSLSLSPGGGGGSGGGGSSYVLTQPSSVSVAPGQTATISCGGHNIGSKNVHWYQQRPGQSPVLVIYQDNKRPSGIPERFSGSNSGNTATLTISGTQAMDEADYYCQVWDNYSVLFGGGTKLTVLGGSGGSQVQLVQSGAEVKKPGESLKVSCKASGYTFTSYYMHWVRQAPGQGLEWMGAIEPMYGSTSYAQKFQGRVTMTRDTSTSTVYMELSSLRSEDTAVYYCARGSAYYYDFADYWGQGTLVTVSSGGSGGSGGSGGSGGSGGSSYVLTQPSSVSVAPGQTATISCGGHNIGSKNVHWYQQRPGQSPVLVIYQDNKRPSGIPERFSGSNSGNTATLTISGTQAMDEADYYCQVWDNYSVLFGGGTKLTVLGGSGGSQVQLVQSGAEVKKPGESLKVSCKASGYTFTSYYMHWVRQAPGQGLEWMGAIEPMYGSTSYAQKFQGRVTMTRDTSTSTVYMELSSLRSEDTAVYYCARGSAYYYDFADYWGQGTLVTVSSAAAGSHHHHHH

SEQ ID NO: 168 - protein, 469 aa, Artificial Sequence
  KiH-scDb-Fc polypeptide chain
EVQLLESGGGLVQPGGSLRLSCAASGFTFSNYDMAWVRQAPGKGLEWVSSISTRGDITSYRDSVKGRFTISRDNSKNTLYLQMNSLRAEDTAVYYCARQDYYTDYMGFAYWGQGTLVTVSSGGGGSGGGGSGGGGSAIQMTQSPSSLSASVGDRVTITCRASEDIYNGLAWYQQKPGKAPKLLIYGASSLQDGVPSRFSGSGSGTEFTLTISSLQPEDEATYYCAGPHKYPLTFGGGTKVEIKDKTHTCPPCPAPEFEGGPSVFLFPPKPKDTLMISRTPEVTCVVVAVSHEDPEVKFNWYVDGVEVHNAKTKPREEQYNSTYRVVSVLTVLHQDWLNGKEYKCKVSNKALPAPIEKTISKAKGQPREPQVYTLPPSREEMTKNQVSLYCLVKGFYPSDIAVEWESNGQPENNYKTTPPVLDSDGSFFLYSKLTVDKSRWQQGNVFSCSVMHEALHNHYTQKSLSLSPG

SEQ ID NO: 169 - protein, 721 aa, Artificial Sequence
  Db-Fc polypeptide chain
SYVLTQPSSVSVAPGQTATISCGGHNIGSKNVHWYQQRPGQSPVLVIYQDNKRPSGIPERFSGSNSGNTATLTISGTQAMDEADYYCQVWDNYSVLFGGGTKLTVLGGSGGSQVQLVQSGAEVKKPGESLKVSCKASGYTFTSYYMHWVRQAPGQGLEWMGAIEPMYGSTSYAQKFQGRVTMTRDTSTSTVYMELSSLRSEDTAVYYCARGSAYYYDFADYWGQGTLVTVSSGGGGSGGGGSDKTHTCPPCPAPEFEGGPSVFLFPPKPKDTLMISRTPEVTCVVVAVSHEDPEVKFNWYVDGVEVHNAKTKPREEQYNSTYRVVSVLTVLHQDWLNGKEYKCKVSNKALPAPIEKTISKAKGQPREPQVYTLPPSREEMTKNQVSLTCLVKGFYPSDIAVEWESNGQPENNYKTTPPVLDSDGSFFLYSKLTVDKSRWQQGNVFSCSVMHEALHNHYTQKSLSLSPGGGGGSGGGGSEVQLLESGGGLVQPGGSLRLSCAASGFTFSNYDMAWVRQAPGKGLEWVSSISTRGDITSYRDSVKGRFTISRDNSKNTLYLQMNSLRAEDTAVYYCARQDYYTDYMGFAYWGQGTLVTVSSGGGGSGGGGSGGGGSAIQMTQSPSSLSASVGDRVTITCRASEDIYNGLAWYQQKPGKAPKLLIYGASSLQDGVPSRFSGSGSGTEFTLTISSLQPEDEATYYCAGPHKYPLTFGGGTKVEIK

SEQ ID NO: 170 - protein, 960 aa, Artificial Sequence
  scDb-mFc polypeptide chain
EVQLLESGGGLVQPGGSLRLSCAASGFTFSNYDMAWVRQAPGKGLEWVSSISTRGDITSYRDSVKGRFTISRDNSKNTLYLQMNSLRAEDTAVYYCARQDYYTDYMGFAYWGQGTLVTVSSGGGGSGGGGSGGGGSAIQMTQSPSSLSASVGDRVTITCRASEDIYNGLAWYQQKPGKAPKLLIYGASSLQDGVPSRFSGSGSGTEFTLTISSLQPEDEATYYCAGPHKYPLTFGGGTKVEIKGGGGSGGGGSAPEFEGGPSVFLFPPKPKDTLMISRTPEVTCVVVAVSHEDPEVKFNWYVDGVEVHNAKTKPREEQYNSTYRVVSVLTVLHQDWLNGKEYKCKVSNKALPAPIEKTISKAKGQPREPQVYTKPPSRDELTKNQVSLSCLVKGFYPSDIAVEWESNGQPENNYKTTVPVLDSDGSFRLASYLTVDKSRWQQGNVFSCSVMHEALHNHYTQKSLSLSPGGGGSGGGGSSYVLTQPSSVSVAPGQTATISCGGHNIGSKNVHWYQQRPGQSPVLVIYQDNKRPSGIPERFSGSNSGNTATLTISGTQAMDEADYYCQVWDNYSVLFGGGTKLTVLGGSGGSQVQLVQSGAEVKKPGESLKVSCKASGYTFTSYYMHWVRQAPGQGLEWMGAIEPMYGSTSYAQKFQGRVTMTRDTSTSTVYMELSSLRSEDTAVYYCARGSAYYYDFADYWGQGTLVTVSSGGSGGSGGSGGSGGSGGSSYVLTQPSSVSVAPGQTATISCGGHNIGSKNVHWYQQRPGQSPVLVIYQDNKRPSGIPERFSGSNSGNTATLTISGTQAMDEADYYCQVWDNYSVLFGGGTKLTVLGGSGGSQVQLVQSGAEVKKPGESLKVSCKASGYTFTSYYMHWVRQAPGQGLEWMGAIEPMYGSTSYAQKFQGRVTMTRDTSTSTVYMELSSLRSEDTAVYYCARGSAYYYDFADYWGQGTLVTVSS

SEQ ID NO: 171 - protein, 960 aa, Artificial Sequence; identical to SEQ ID NO: 170
  Bi-scFv-Fc polypeptide chain

SEQ ID NO: 172 - protein, 8 aa, Homo sapiens
SFFPPGYQ

SEQ ID NO: 173 - protein, 725 aa, Artificial Sequence
  scFv-Ig polypeptide chain
QVQLVQSGAEVKKPGSSVKVSCKASGGTFSSYTISWVRQAPGQGLEWMGGIIPIFGTANYAQKFQGRVTITADESTSTAYMELSSLRSEDTAVYYCARGGSSGWWWGQGTLVTVSSASTKGPSVFPLAPSSKSTSGGTAALGCLVKDYFPEPVTVSWNSGALTSGVHTFPAVLQSSGLYSLSSVVTVPSSSLGTQTYICNVNHKPSNTKVDKKVEPKSCDKTHTCPPCPAPEFEGGPSVFLFPPKPKDTLMISRTPEVTCVVVAVSHEDPEVKFNWYVDGVEVHNAKTKPREEQYNSTYRVVSVLTVLHQDWLNGKEYKCKVSNKALPAPIEKTISKAKGQPREPQVYTLPPSREEMTKNQVSLTCLVKGFYPSDIAVEWESNGQPENNYKTTPPVLDSDGSFFLYSKLTVDKSRWQQGNVFSCSVMHEALHNHYTQKSLSLSPGGGGGSGGGGSGGGGSGGGGSGGGGSGGGGSDIQMTQSPASLSASVGETVTITCRVSENIYSYLAWYQQKQGKSPQLLVYNAKTLAEGVPSRFSGSGSGTQFSLKINSLQPEDFGSYYCQHHYGTPWTFGGGTKLEIKGGSGGSGGSGGSGGSGGSGGSEVQLQESGPGLVKPSQSLSLTCTVTGYSITSDYAWNWIRQFPGNKLEWMGYITYSGSTSYNPSLESRISITRDTSTNQFFLQLNSVTTEDTATYYCARGGYYGSSWGVFAYWGQGTLVTVSA

SEQ ID NO: 174 - protein, 216 aa, Artificial Sequence
  scFv-Ig polypeptide chain
QSVLTQPPSASGTPGQRVIISCSGSHSNIGSNNVNWYQQLPGTAPKLLIYNNNQRPSGVPDRFSGSKSGTSASLAISGLQSEDESDYFCGTWDDSLNGPVFGGGTKLTVLGQPKAAPSVTLFPPSSEELQANKATLVCLISDFYPGAVTVAWKADSSPVKAGVETTTPSKQSNNKYAASSYLSLTPEQWKSHRSYSCQVTHEGSTVEKTVAPTECS

SEQ ID NO: 175 - protein, 727 aa, Artificial Sequence
  scFv-Ig polypeptide chain
QVQLVQSGAEVKKPGSSVKVSCKASGGTFSSYTISWVRQAPGQGLEWMGGIIPIFGTANYAQKFQGRVTITADESTSTAYMELSSLRSEDTAVYYCARGGSSGWWWGQGTLVTVSSASTKGPSVFPLAPSSKSTSGGTAALGCLVKDYFPEPVTVSWNSGALTSGVHTFPAVLQSSGLYSLSSVVTVPSSSLGTQTYICNVNHKPSNTKVDKKVEPKSCDKTHTCPPCPAPEFEGGPSVFLFPPKPKDTLMISRTPEVTCVVVAVSHEDPEVKFNWYVDGVEVHNAKTKPREEQYNSTYRVVSVLTVLHQDWLNGKEYKCKVSNKALPAPIEKTISKAKGQPREPQVYTLPPSREEMTKNQVSLTCLVKGFYPSDIAVEWESNGQPENNYKTTPPVLDSDGSFFLYSKLTVDKSRWQQGNVFSCSVMHEALHNHYTQKSLSLSPGGGGGSGGGGSGGGGSGGGGSGGGGSGGGGSQSALTQPASVSGSPGQSITISCSGSSSNIGNNAVNWYQQLPGKAPKLLIYYDDLLPSGVSDRFSGSKSGTSAFLAISGLQSEDEADYYCAAWDDSLNGPVFGGGTKLTVLGGSGGSGGSGGSGGSGGSGGSQVQLVESGGGLVKPGGSLRLSCAASGFTFSSYGMHWVRQAPGKGLEWVAFIRYDGSNKYYADSVKGRFTISRDNSKNTLYLQMNSLRAEDTAVYYCAKDRGLGDGTYFDYWGQGTTVTVSS

SEQ ID NO: 176 - protein, 216 aa, Artificial Sequence; identical to SEQ ID NO: 174
  scFv-Ig polypeptide chain

SEQ ID NO: 177 - protein, 722 aa, Artificial Sequence
  scFv-Ig polypeptide chain
QVQLVQSGAEVKKPGSSVKVSCKASGGTFSSYTISWVRQAPGQGLEWMGGIIPIFGTANYAQKFQGRVTITADESTSTAYMELSSLRSEDTAVYYCARGGSSGWWWGQGTLVTVSSASTKGPSVFPLAPSSKSTSGGTAALGCLVKDYFPEPVTVSWNSGALTSGVHTFPAVLQSSGLYSLSSVVTVPSSSLGTQTYICNVNHKPSNTKVDKKVEPKSCDKTHTCPPCPAPEFEGGPSVFLFPPKPKDTLMISRTPEVTCVVVAVSHEDPEVKFNWYVDGVEVHNAKTKPREEQYNSTYRVVSVLTVLHQDWLNGKEYKCKVSNKALPAPIEKTISKAKGQPREPQVYTLPPSREEMTKNQVSLTCLVKGFYPSDIAVEWESNGQPENNYKTTPPVLDSDGSFFLYSKLTVDKSRWQQGNVFSCSVMHEALHNHYTQKSLSLSPGGGGGSGGGGSGGGGSGGGGSGGGGSGGGGSSYVLTQPSSVSVAPGQTATISCGGHNIGSKNVHWYQQRPGQSPVLVIYQDNKRPSGIPERFSGSNSGNTATLTISGTQAMDEADYYCQVWDNYSVLFGGGTKLTVLGGSGGSGGSGGSGGSGGSGGSQVQLVQSGAEVKKPGESLKVSCKASGYTFTSYYMHWVRQAPGQGLEWMGAIEPMYGSTSYAQKFQGRVTMTRDTSTSTVYMELSSLRSEDTAVYYCARGSAYYYDFADYWGQGTLVTVSS

SEQ ID NO: 178 - protein, 216 aa, Artificial Sequence; identical to SEQ ID NO: 174
  scFv-Ig polypeptide chain